European Patent Application EP 4 148 145 A1, published March 15, 2023. Title: Method for Spatial Tagging and Analysing Nucleic Acids in a Biological Specimen. Applicant: Spatial Transcriptomics AB. The sequence listing filed with the application follows.

SEQUENCE LISTING (8 sequences)

SEQ ID NO: 1 - DNA, 1680 bp, Murine leukemia virus
  source 1..1680: mol_type = genomic DNA
gcttttcccctcgagcgcccagactgggattacaccacccaggcaggtaggaaccacctagtccactatcgccagttgctcctagcgggtctccaaaacgcgggcagaagccccaccaatttggccaaggtaaaagggataacacagggacctaatgagtctccctcagcctttttagagagactcaaggaggcctatcgcaggtacactccttatgaccctgaggacccagggcaagaaaccaatgtgtctatgtcattcatctggcagtctgccccggatatcgggcgaaagttagggcggttagaagatttaaagagcaagaccttaggagacttagttagggaggctgaaaagatctttaataaacgtgaaaccccggaagaaagagaggaacgtatcaggagagaaacagaggaaaaagaagaacgccgtaggacagtggatgagcagaaagagaaagaaagggaccgcagaagacatagagagatgagcaagctcttggccactgtagttattggtcaggaacaggatagacaggagggagagcggaagaggccccaacttgataaggatcaatgcgcctactgcaaagaaaaggggcactgggctaaagactgtcccaagaagccacgagggccccgaggacccaggccccagacctccctcctgaccttaggtgactagggaggtcagggtcaggaccccccccctgaacccaggataaccctcaaagtcggggggcaacccgtcaccttcctggtagatactggggcccaacactccgtgctgacccaaaatcctggacccctaagtgacaagtctgcctgggtccaaggggctactggaggaaagcggtatcgctggaccacggatcgcaaagtgcatctagctaccggtaaggtcacccactctttcctccatgtaccagactgcccctatcctctgctaggaagagatttgctgactaaactaaaagcccaaatccactttgagggatcaggagctcaggttgtgggaccaatgggacagcccctgcaagtgctgaccctaaacatagaagatgagtatcggctacatgagacctcaaaagagccggatgtttctctagggttcacatggctttctgattttcctcaggcctgggcggaatccgggggcatgggactggcagttcgccaagctcctctgatcatacctctgaaggcaacctctacccccgtgtccataaaacaataccccatgtcacaagaagccagactggggatcaagccccacatacagagactgttggaccagggaatactggtaccctgccagtccccctggaacacgcccctgctacccgttaagaaaccagggactaatgattacaggcctgtccaagatctgagagaagtcaacaagcgggtggaagacatccaccccaccgtgcccaacccttacaacctcttgagcgggctcccaccgtcccaccagtggtacactgtgcttgacttaaaggatgcctttttctgcctgagactccaccccaccagtcagcctctcttcgcctttgagtggagagacccagagatgggaatctcaggacaattaacctggaccagactcccacagggtttcaaaaacagtcccaccctgtttgatgaggcactgcacagagacctagcagacttccgg

SEQ ID NO: 2 - protein, 560 aa, Murine leukemia virus
  SITE 229: note = misc_feature - Xaa can be any naturally occurring amino acid
AFPLERPDWDYTTQAGRNHLVHYRQLLLAGLQNAGRSPTNLAKVKGITQGPNESPSAFLERLKEAYRRYTPYDPEDPGQETNVSMSFIWQSAPDIGRKLGRLEDLKSKTLGDLVREAEKIFNKRETPEEREERIRRETEEKEERRRTVDEQKEKERDRRRHREMSKLLATVVIGQEQDRQEGERKRPQLDKDQCAYCKEKGHWAKDCPKKPRGPRGPRPQTSLLTLGDXGGQGQDPPPEPRITLKVGGQPVTFLVDTGAQHSVLTQNPGPLSDKSAWVQGATGGKRYRWTTDRKVHLATGKVTHSFLHVPDCPYPLLGRDLLTKLKAQIHFEGSGAQVVGPMGQPLQVLTLNIEDEYRLHETSKEPDVSLGFTWLSDFPQAWAESGGMGLAVRQAPLIIPLKATSTPVSIKQYPMSQEARLGIKPHIQRLLDQGILVPCQSPWNTPLLPVKKPGTNDYRPVQDLREVNKRVEDIHPTVPNPYNLLSGLPPSHQWYTVLDLKDAFFCLRLHPTSQPLFAFEWRDPEMGISGQLTWTRLPQGFKNSPTLFDEALHRDLADFR

SEQ ID NO: 3 - DNA, 100 bp, synthetic construct
  misc_feature 1..100: note = Probe 1
  misc_feature 72..73: note = n is a, c, g, t or u
  misc_feature 76..77: note = n is a, c, g, t or u
  misc_feature 100: note = n is a, c, g, t or u
  source 1..100: mol_type = other DNA
  misc_feature 1..5: note = RNA
tttttgactcgtaatacgactcactatagggacacgacgctcttccgatctgtccgatatgattgccgcwsnnwsnnvttttttttttttttttttttvn

SEQ ID NO: 4 - DNA, 35 bp, synthetic construct
  misc_feature 1..35: note = Ligation adaptor
  source 1..35: mol_type = other DNA
agatcggaagagcacacgtctgaactccagtcacc

SEQ ID NO: 5 - DNA, 30 bp, synthetic construct
  misc_feature 1..30: note = Second reverse transcription primer
  source 1..30: mol_type = other DNA
tgactggagttcagacgtgtgctcttccga

SEQ ID NO: 6 - DNA, 57 bp, synthetic construct
  misc_feature 1..57: note = PCR primer InPE1.0
  source 1..57: mol_type = other DNA
atgatacggcgaccaccgagatctacactctttccctacacgacgctcttccgatct

SEQ ID NO: 7 - DNA, 34 bp, synthetic construct
  misc_feature 1..34: note = PCR primer InPE2.0
  source 1..34: mol_type = other DNA
gtgactggagttcagacgtgtgctcttccgatct

SEQ ID NO: 8 - DNA, 42 bp, synthetic construct
  misc_feature 1..42: note = PCR Index primer
  misc_feature 24..29: note = n is a, c, g, or t
  source 1..42: mol_type = other DNA
aagcagaagacggcatacgagatnnnnnngtgactggagttc